European Patent Application EP 4 692 312 A1, published February 11, 2026. Title: L-GLUTAMIC ACID-PRODUCING BACTERIUM AND METHOD FOR PRODUCING L-GLUTAMIC ACID. Applicant: Ajinomoto Co., Inc. Application WO PCT/JP2023/047150, filed December 28, 2023. The sequence listing filed with the application follows.

SEQUENCE LISTING (10 sequences)

SEQ ID NO: 1 - DNA, 1380 bp, Corynebacterium glutamicum
  source 1..1380: mol_type = genomic DNA
atgcttgtgggcgtacctgtcccgcgagtgaggtcttacgcgcgggattcgtcttgtgaaaggttagctgacctgatgaccgatgcccaccaagcggacgatgtccgttaccagccactgaacgagcttgatcctgaggtggctgctgccatcgctggggaacttgcccgtcaacgcgatacattagagatgatcgcgtctgagaacttcgttccccgttctgttttgcaggcgcagggttctgttcttaccaataagtatgccgagggttaccctggccgccgttactacggtggttgcgaacaagttgacatcattgaggatcttgcacgtgatcgtgcgaaggctctcttcggtgcagagttcgccaatgttcagcctcactctggcgcacaggctaatgctgctgtgctgatgactttggctgagccaggcgacaagatcatgggtctgtctttggctcatggtggtcacttgacccacggaatgaagttgaacttctccggaaagctgtacgaggttgttgcgtacggtgttgatcctgagaccatgcgtgttgatatggatcaggttcgtgagattgctctgaaggagcagccaaaggtaattatcgctggctggtctgcataccctcgccaccttgatttcgaggctttccagtctattgctgcggaagttggcgcgaagctgtgggtcgatatggctcacttcgctggtcttgttgctgctggtttgcacccaagcccagttccttactctgatgttgtttcttccactgtccacaagactttgggtggacctcgttccggcatcattctggctaagcaggagtacgcgaagaagctgaactcttccgtattcccaggtcagcagggtggtcctttgatgcacgcagttgctgcgaaggctacttctttgaagattgctggcactgagcagttccgtgaccgtcaggctcgcacgttggagggtgctcgcattcttgctgagcgtctgactgcttctgatgcgaaggccgctggcgtggatgtcttgaccggtggcactgatgtgcacttggttttggctgatctgcgtaactcccagatggatggccagcaggcggaagatctgctgcacgaggttggtatcactgtgaaccgtaacgcggttcctttcgatcctcgtccaccaatggttacttctggtctgcgtattggtactcctgcgctggctacccgtggtttcgatattcctgcattcactgaggttgcagacatcattggtactgctttggctaatggtaagtccgcagacattgagtctctgcgtggccgtgtagcaaagcttgctgcagattacccactgtatgagggcttggaagactggaccatcgtctaa

SEQ ID NO: 2 - protein, 459 aa, Corynebacterium glutamicum
MLVGVPVPRVRSYARDSSCERLADLMTDAHQADDVRYQPLNELDPEVAAAIAGELARQRDTLEMIASENFVPRSVLQAQGSVLTNKYAEGYPGRRYYGGCEQVDIIEDLARDRAKALFGAEFANVQPHSGAQANAAVLMTLAEPGDKIMGLSLAHGGHLTHGMKLNFSGKLYEVVAYGVDPETMRVDMDQVREIALKEQPKVIIAGWSAYPRHLDFEAFQSIAAEVGAKLWVDMAHFAGLVAAGLHPSPVPYSDVVSSTVHKTLGGPRSGIILAKQEYAKKLNSSVFPGQQGGPLMHAVAAKATSLKIAGTEQFRDRQARTLEGARILAERLTASDAKAAGVDVLTGGTDVHLVLADLRNSQMDGQQAEDLLHEVGITVNRNAVPFDPRPPMVTSGLRIGTPALATRGFDIPAFTEVADIIGTALANGKSADIESLRGRVAKLAADYPLYEGLEDWTIV

SEQ ID NO: 3 - DNA, 1380 bp, Corynebacterium glutamicum
  source 1..1380: mol_type = genomic DNA
atgcttgtgggcgtacctgtcccgcgagtgaggtcttacgcgcgggattcgtcttgtgaaaggttagctgacctgatgaccgatgcccaccaagcggacgatgtccgttaccagccactgaacgagcttgatcctgaggtggctgctgccatcgctggggaacttgcccgtcaacgcgatacattagagatgatcgcgtctgagaacttcgttccccgttctgttttgcaggcgcagggttctgttcttaccaataagtatgccgagggttaccctggccgccgttactacggtggttgcgaacaagttgacatcattgaggatcttgcacgtgatcgtgcgaaggctctcttcggtgcagagttcgccaatgttcagcctcactctggcgcacaggctaatgctgctgtgctgatgactttggctgagccaggcgacaagatcatgggtctgtctttggctcatggtggtcacttgacccacggaatgaagttgaacttctccggaaagctgtacgaggttgttgcgtacggtgttgatcctgagaccatgcgtgttgatatggatcaggttcgtgagattgctctgaaggagcagccaaaggtaattatcgctggctggtctgcataccctcgccaccttgatttcgaggctttccagtctattgctgcggaagttggcgcgaagctgtgggtcgatatggctcacttcgctggtcttgttgctgctggtttgcacccaagcccagttccttactctgatgttgtttcttccactgtccacaagactttgagtggacctcgttccggcatcattctggctaagcaggagtacgcgaagaagctgaactcttccgtattcccaggtcagcagggtggtcctttgatgcacgcagttgctgcgaaggctacttctttgaagattgctggcactgagcagttccgtgaccgtcaggctcgcacgttggagggtgctcgcattcttgctgagcgtctgactgcttctgatgcgaaggccgctggcgtggatgtcttgaccggtggcactgatgtgcacttggttttggctgatctgcgtaactcccagatggatggccagcaggcggaagatctgctgcacgaggttggtatcactgtgaaccgtaacgcggttcctttcgatcctcgtccaccaatggttacttctggtctgcgtattggtactcctgcgctggctacccgtggtttcgatattcctgcattcactgaggttgcagacatcattggtactgctttggctaatggtaagtccgcagacattgagtctctgcgtggccgtgtagcaaagcttgctgcagattacccactgtatgagggcttggaagactggaccatcgtctaa

SEQ ID NO: 4 - protein, 459 aa, Corynebacterium glutamicum
MLVGVPVPRVRSYARDSSCERLADLMTDAHQADDVRYQPLNELDPEVAAAIAGELARQRDTLEMIASENFVPRSVLQAQGSVLTNKYAEGYPGRRYYGGCEQVDIIEDLARDRAKALFGAEFANVQPHSGAQANAAVLMTLAEPGDKIMGLSLAHGGHLTHGMKLNFSGKLYEVVAYGVDPETMRVDMDQVREIALKEQPKVIIAGWSAYPRHLDFEAFQSIAAEVGAKLWVDMAHFAGLVAAGLHPSPVPYSDVVSSTVHKTLSGPRSGIILAKQEYAKKLNSSVFPGQQGGPLMHAVAAKATSLKIAGTEQFRDRQARTLEGARILAERLTASDAKAAGVDVLTGGTDVHLVLADLRNSQMDGQQAEDLLHEVGITVNRNAVPFDPRPPMVTSGLRIGTPALATRGFDIPAFTEVADIIGTALANGKSADIESLRGRVAKLAADYPLYEGLEDWTIV

SEQ ID NO: 5 - DNA, 37 bp, Corynebacterium glutamicum
  source 1..37: mol_type = other DNA
ccaagcttgcatgccatgcttgtgggcgtacctgtcc

SEQ ID NO: 6 - DNA, 37 bp, Corynebacterium glutamicum
  source 1..37: mol_type = other DNA
cggtacccggggatcttagacgatggtccagtcttcc

SEQ ID NO: 7 - DNA, 1602 bp, Corynebacterium glutamicum
  source 1..1602: mol_type = genomic DNA
atgattttaggcgtacccattcaatatttgctctattcattgtggaattggattgtcgataccggttttgatgtagcaattatcctggtcttggcgtttttgattccacgtatcggccgactggccatgcgtattatcaagcagcgagtggagtctgcagccgatgcggacaccactaagaaccagctcgcgttcgctggcgttggcgtttatatcgcgcaaattgtggcgtttttcatgcttgccgtctccgcgatgcaggcttttggtttctctctcgcgggcgctgcgattccggcaaccattgcgtcagctgccattggtcttggtgcgcagtcgattgttgcggacttcttggccggatttttcatcctgacggaaaagcaattcggcgtgggtgactgggtgcgctttgagggcaacggcatcgttgttgaaggcaccgtcattgagatcaccatgcgcgcgaccaaaattcgcacgattgcacaagagaccgtgatcatcccgaactccacggcgaaagtgtgcatcaacaattctaataactggtcgcgtgcggttgtcgttattccgatccccatgttgggttctgaaaacatcacagatgtcatcgcgcgctctgaagctgcgactcgtcgcgcacttggccaggagaaaatcgcaccggaaatcctcggtgaactcgatgtgcacccagccacggaagtcacaccgccaacggtggtcggcatgccgtggatggtcaccatgcgtttcctcgtgcaagtcaccgccggcaatcaatggctggtcgaacgcgccatccgcacagaaatcatcaacgaattctgggaagaatacggcagcgcaaccactacatcgggaaccctcattgattccttacacgttgagcatgaagagccaaagacctcgcttatcgacgcctccccccaggctcttaaggaaccgaagccggaggctgcggcgacggttgcatcgctagctgcatcgtctaacgacgatgcagacaatgcagacgcctcggcgatcaatgcaggcaatccagagaaggaacttgattccgatgtgctggaacaagaactctccagcgaagaaccggaagaaacagcaaaaccagatcactctctccgaggcttcttccgcactgattactacccaaatcggtggcagaagatcctgtcgtttggcggacgtgtccgcatgagcacttccctgttgttgggtgcgctgctcttgctgtcactatttaaggtcatgactgtggaaccaagtgagaattggcaaaactccagtggatggctgtcaccaagcactgccacctcaactgcggtgaccacctccgaaacttccgcgccagcaagcacgccttcgatgacagtgcccactacggtggaggagaccccaacgatggaatctagcgtcgaaacgcagcaggaaacctcaacccctgcaaccgcaacgccccagcgagccgacaccatcgaaccgaccgaggaagccacgtcgcaggaggaaacgactgcatcgcagacgcagtctccagcagtggaagcaccaaccgcggtccaagaaacagttgcgccgacgtccaccccttag

SEQ ID NO: 8 - protein, 533 aa, Corynebacterium glutamicum
MILGVPIQYLLYSLWNWIVDTGFDVAIILVLAFLIPRIGRLAMRIIKQRVESAADADTTKNQLAFAGVGVYIAQIVAFFMLAVSAMQAFGFSLAGAAIPATIASAAIGLGAQSIVADFLAGFFILTEKQFGVGDWVRFEGNGIVVEGTVIEITMRATKIRTIAQETVIIPNSTAKVCINNSNNWSRAVVVIPIPMLGSENITDVIARSEAATRRALGQEKIAPEILGELDVHPATEVTPPTVVGMPWMVTMRFLVQVTAGNQWLVERAIRTEIINEFWEEYGSATTTSGTLIDSLHVEHEEPKTSLIDASPQALKEPKPEAAATVASLAASSNDDADNADASAINAGNPEKELDSDVLEQELSSEEPEETAKPDHSLRGFFRTDYYPNRWQKILSFGGRVRMSTSLLLGALLLLSLFKVMTVEPSENWQNSSGWLSPSTATSTAVTTSETSAPASTPSMTVPTTVEETPTMESSVETQQETSTPATATPQRADTIEPTEEATSQEETTASQTQSPAVEAPTAVQETVAPTSTP

SEQ ID NO: 9 - DNA, 3060 bp, Corynebacterium glutamicum
  source 1..3060: mol_type = genomic DNA
atgattttaggcgtacccattcaatatttgctctattcattgtggaattggattgtcgataccggttttgatgtagcaattatcctggtcttggcgtttttgattccacgtatcggccgactggccatgcgtattatcaagcagcgagtggagtctgcagccgatgcggacaccactaagaaccagctcgcgttcgctggcgttggcgtttatatcgcgcaaattgtggcgtttttcatgcttgccgtctccgcgatgcaggcttttggtttctctctcgcgggcgctgcgattccggcaaccattgcgtcagctgccattggtcttggtgcgcagtcgattgttgcggacttcttggccggatttttcatcctgacggaaaagcaattcggcgtgggtgactgggtgcgctttgagggcaacggcatcgttgttgaaggcaccgtcattgagatcaccatgcgcgcgaccaaaattcgcacgattgcacaagagaccgtgatcatcccgaactccacggcgaaagtgtgcatcaacaattctaataactggtcgcgtgcggttgtcgttattccgatccccatgttgggttctgaaaacatcacagatgtcatcgcgcgctctgaagctgcgactcgtcgcgcacttggccaggagaaaatcgcaccggaaatcctcggtgaactcgatgtgcacccagccacggaagtcacaccgccaacggtggtcggcatgccgtggatggtcaccatgcgtttcctcgtgcaagtcaccgccggcaatcaatggctggtcgaacgcgccatccgcacagaaatcatcaacgaattctgggaagaatacggcagcgcaaccactacatcgggaaccctcattgattccttacacgttgagcatgaagagccaaagacctcgcttatcgacgcctccccccaggctcttaaggaaccgaagccggaggctgcggcgacggttgcatcgctagctgcatcgtctaacgacgatgcagacaatgcagacgcctcggcgatcaatgcaggcaatccagagaaggaacttgattccgatgtgctggaacaagaactctccagcgaagaaccggaagaaacagcaaaaccagatcactctctccgaggcttcttccgcactgattactacccaaatcggtggcagaagatcctgtcgtttggcggacgtgtccgcatgagcacttccctgttgttgggtgcgctgctcttgctgtcactatttaaggggctcttcctgttttagagtgcattgatcttatggaccaactgccctgaatggataaggcaccgcagaatgtagtggttcaaattacggaaacctagagcaatcccacgcaaatgctccaaccgtccgttgatcgcttcgaccggaccgttggagacaccaacatcgaaatacgccaacacatcaccaagtcgtttaaacaaactacgacccaactgcgcgagttccttattcggccccttcaacacccgaagctgatcaataatggtccgcattttcttcttcgcttcacgcttattacccatctgataacaatcaataatcgcctgatacgcaagccacgcaagctttaacaccccgtagtctttgtcatacgcccacaactgctccaagctttcttgctgacgaggactcaaccacttgtgcgtggtcaacaaggtcttccggtttttatacaacggatcctggcttaaaccacgacgctggtatttctcccgctggaggcgttgccggcaggcggtgagcttgtcaccagcaagccgcacaacatggaatggatccatcacgcgacgagcagaaggaatgagttctttacttgctgtggcgtagccttggaacccatccatggacacgatccgtatctgattgcggaactgttcaccgcgggaaccaagccaggaccgtaaagcatcagcactacgacctgggacgacatctaataaccgggcaggacaccgtgagtcataccgatgcccggtcatatcgacaatcacggtgacaaacccatcaccatgcttagccctattatgtgaccacttatgctcatccaccccaatgacatacactccatcaagatggtgaggatcgttatagaccagctcacggcacatatcgagggctagttggcaggttaaatcccaccctagcccaagtgctttcgcggttgcgtgaacactcatccggtcaatagcaaggcgttgcaaaatccagcgggtgacccggtgggtgacctttttaccgtggtcagcgcagcttagttctgcttggaaatacttttgcttacatgtcgggttggtgcagcggtagcgaggtagacggataaacagtttggtgggaaacccgacgatgggtaaatcaatgagcatccggtgggtgtgatgacgaaacaccccaggttgggagcattctgggcaggtggaggtatagtcgagtgcgtctgcttcgatcagggtgtaatcacctgcatcggaagcgccggtgatggtgagtcctagttccgcagtgcggcagatggtgtcagcgatgatgttgccggtagacttcatgggtagagccttttgttggtgtttggttagcttagatacctaaaccttaaccctgacaaaaggctcgtttattttcgggtctacaccgctagcccaggttctgtgatgtaccccaaaaccggaagggccatttaaggtcatgactgtggaaccaagtgagaattggcaaaactccagtggatggctgtcaccaagcactgccacctcaactgcggtgaccacctccgaaacttccgcgccagcaagcacgccttcgatgacagtgcccactacggtggaggagaccccaacgatggaatctagcgtcgaaacgcagcaggaaacctcaacccctgcaaccgcaacgccccagcgagccgacaccatcgaaccgaccgaggaagccacgtcgcaggaggaaacgactgcatcgcagacgcagtctccagcagtggaagcaccaaccgcggtccaagaaacagttgcgccgacgtccacccct

SEQ ID NO: 10 - protein, 423 aa, Corynebacterium glutamicum
MILGVPIQYLLYSLWNWIVDTGFDVAIILVLAFLIPRIGRLAMRIIKQRVESAADADTTKNQLAFAGVGVYIAQIVAFFMLAVSAMQAFGFSLAGAAIPATIASAAIGLGAQSIVADFLAGFFILTEKQFGVGDWVRFEGNGIVVEGTVIEITMRATKIRTIAQETVIIPNSTAKVCINNSNNWSRAVVVIPIPMLGSENITDVIARSEAATRRALGQEKIAPEILGELDVHPATEVTPPTVVGMPWMVTMRFLVQVTAGNQWLVERAIRTEIINEFWEEYGSATTTSGTLIDSLHVEHEEPKTSLIDASPQALKEPKPEAAATVASLAASSNDDADNADASAINAGNPEKELDSDVLEQELSSEEPEETAKPDHSLRGFFRTDYYPNRWQKILSFGGRVRMSTSLLLGALLLLSLFKGLFLF